European Patent Application EP 4 763 991 A1, published June 24, 2026. Title: 利用生物酶法高效制备莱鲍迪苷M的方法. Applicant: 桂林莱茵生物科技股份有限公司. The sequence listing filed with the application follows.

SEQUENCE LISTING (20 sequences)

SEQ ID NO: 1 - protein, 458 aa, Coffea arabica
MEENQTISSILMLPWLAHGHVSPYLELARKLTARNFNIYLCSTPINLSSIRSKISPKFGKSIQLIELNLPTLPNLPPQYHTTNGLPPHLMVTLKEAFEMASPNFCKILRTLMPDLLIYDLLQPWAPEAASYYNIPAVEFITCSATMTSCMLHFFRTPGIQFPYSSTIFFRDYESAIANKLLERDEDANRVAQCIERSSKILLIKSFKEIEGKYNDYVSCLSGKKVVPVGPLVQDPVHDNEDLTIMEWLNTKGKYSTVFVSFGSEYFLSKGDLEGVAHGLELSSVNFVWVVRFPKGENIIVEEALPKGFLKRVGERGKIVNGWAPQAKILNHSSIGGFVSHCGWNSVLEGMRFGVPIIAVPMHLDQPVNARLLQEVGAGMEVVRGSTGKIHGENMAEIINQVVKGPRGEPVRKKARDLRETLELKGDEEIDEVVKELVQLCLTEDKNNGLHLEHHHHHH

SEQ ID NO: 2 - protein, 825 aa, Capsicum annuum
MDASMAINEKSLSVLMFPWLGHGHVSPFLELAKKLVTRNFIIFLCSTPANLKSIKQKLINENLTQKIHLIEIHLPCLTDLPPHYHTTNGLPPHLMSTLKKAFAMSRPIFTQILNAIEPDLLLYDLLQPWAPKVAAEKNIPSVCFVTSSATMFSYMFHNFQNPNLVFPYPSIYYRDYELARMIKNKDLESIEQQKKDDTSVKLCFKRSSNIVLIKGFKELDGKYCDYISSLTNKRVVPVGPLVQEPTSDVDNSLILKWLNQKSKGSTVFVSFGSEYFLSQEDREEIAHGLEQSRVNFVWVVRFPKGEKLKLEQALPLGFFKKVGERGMVVEDWAPQAKILAHPNIGGFVSHCGWNSVMESMKIGVPIIAMPMHLDQPLNARLVEEVGVGLEVVRDKNGKLERETISQVINKVVLGKEGEPIRAKAKKMSATLGVKGDEEIDDVVQELVKLCKKSKSIRAIIVKQNMVLKRMESDGPKSGSGCRIENGGSGSLVNKSNVNEEYVEALRTKSYVELYNKVQEQLEEGRLNDDYKLSSSSSLQLDTNLCQEEISELPESVKLHPLIVNYFDITLEACRICELLLQNVHQTRANYKKIRRAIGLMKIEQDSMHCYRVYRELASFASLNNSFSVVNQVQILDTREGHDSLLQKLSSQFRRVKRRMKFWKSCKRVFGISIVIGYIGVMIALLVLALHSMVCIVAAPGLIACSYKVFKRRLKTDKKEESSSSQERLIAQLDVAAKGMYILINDFDTISRLVRRLYDEIEHNRSVAEMCTRKKNTDMLKEAIRDYSINKNCFIEQLKELEEHICLCFVTINRSRRMVLQEVVSK

SEQ ID NO: 3 - protein, 462 aa, Coffea arabica
MEENQTISSILMLPWLAHGHVSPYLELAKKLTARNFNIYLCSTPINLSSIRSKISPKFGKSIQLIELNLPTLPNLPPQYHTTNGLPPHLMVTLKEAFEMASPNFCKILRTLMPDLLIYDLLQPWAPEAASYYNIPAVEFITCSATMTSCMLHFFQTPGIQFPYSSTIFFRDYESAIANKLLERDGDANRVAQCIERSSKVLLIKSFKEIEGKYNDYVSCLSGKKVVPVGPLVQDPVHDNEDSTIMEWLNTKGKYSTVFVSFGSEYFLSKEDLEGVAHGLELSSLNFVWVVRFPKGENIIVEEALPKGFLKRVGERGKIVNGWAPQAKILNHSSIGGFVSHCGWNSVLEGMRFGVPIIAVPMHLDQPVNARLLEEVGAGMEVVRGSTGKIHGEDMAEIINQVVKGPRGEPVRKKARDLREKLELKGDEEIDEVVKELVQLCLTKDKSNGLHQPIQLEHHHHHH

SEQ ID NO: 4 - protein, 459 aa, Coffea eugenioides
MENHATFNVLMLPWLAHGHVSPYLELAKKLTARNFNVYLCSSPATLSSVRSKLTEKFSQSIHLVELHLPKLPELPAEYHTTNGLPPHLMPTLKDAFDMAKPNFCNVLKSLKPDLLIYDLLQPWAPEAASAFNIPAVVFISSSATMTSFGLHFFKNPGTKYPYGNAIFYRDYESVFVENLTRRDRDTYRVINCMERSSKIILIKGFNEIEGKYFDYFSCLTGKKVVPVGPLVQDPVLDDEDCEIMQWLNKKEKVSTVFVSFGSEYFLSKKDMEEIAHGLELSNVDFIWVVRFPKGENIVIEETLPKGFFERVGERGLVVNGWAPQAKILTHPNVGGFVSHCGWNSVMESMKFGLPIIAMPMHLDQPINARLIEEVGAGVEVLRDSKGKLHRERMAETINKVMKEASGESVRKKARELQEKMDLKGDEEIDDVVKELVQLCATKNKRNGLHYYLEHHHHHH

SEQ ID NO: 5 - protein, 460 aa, Coffea canephora
MENHATFNVLMLPWLAHGHVSPYLELAMKLTARNFNVYLCSSPATLSSVRSKLTEKFSQSIHLVELHLPKLPELPAEYHTTNGLPPHLMPTLKDAFDMAKPNFCNVLKSLKPDLLIYDLLQPWAPEAASAFNIPAVVFISSSATMTSFGLHFFKNPGTKYPYGNTIFYRDYESVFVENLKKRDRDTYRVVNCMERSSKIILIKGFKEIEGKYFDYFSCLTGKKVVPVGPLVQDPVLDDEDCRIMQWLNKKEKGSTVFVSFGSEYFLSKEDMEEIAHGLELSNVDFIWVVRFPKGENIVIEETLPKGFFERVGERGLVVNGWAPQAKILTHPNVGGFVSHCGWNSVMESMKFGLPIVAMPMHLDQPINARLIEEVGAGVEVLRDSKGKLHRERMAETINKVTKEASGEPARKKARELQEKLELKGDEEIDDVVKELVQLCATKNKRNGLHCYNLEHHHHHH

SEQ ID NO: 6 - protein, 459 aa, Coffea arabica
MENHATFNVLMLPWLAHGHVSPYLELAKKLTARNFNVYLCSSPATLSSVRSKLTEKFSQSIHLVELHLPKLPELPAEYHTTNGLPPHLMPTLKDAFDMAKPNFCNVLKSLKPDLLIYDLLQPWAPEAASAFNIPAVVFISSSATMTSFGLHFFKNPGTKYPYGNAIFYRDYESVFVENLTRRDRDTYRVINCMERSSKIILIKGFNEIEGKYFDYFSCLTGKKVVPVGPLVQDPVLDDEDCRIMQWLNKKEKGSTVFVSFGSEYFLSKKDMEEIAHGLEVSNVDFIWVVRFPKGENIVIEETLPKGFFERVGERGLVVNGWAPQAKILTHPNVGGFVSHCGWNSVMESMKFGLPIIAMPMHLDQPINARLIEEVGAGVEVLRDSKGKLHRERMAETINKVMKEASGESVRKKARELQEKLELKGDEEIDDVVKELVQLCATKNKRNGLHYYLEHHHHHH

SEQ ID NO: 7 - protein, 458 aa, Coffea eugenioides
MEENQTISSILMLPWLAHGHVSPYLELARKLTARNFNIYLCSTPINLSSIRSKISPKFGKSIQLIELNLPTLPNLPPQYHTTNGLPPHLMVTLKEAFEMASPNFCKILRTLMPDLLIYDLLQPWAPEAASYYNIPAVEFITCSATMTSCMLHFFRTPGIQFPYSSTIFFRDYESAIANKLLERDEDANRVAQCIERSSKILLIKSFKEIEGKYNDYVSCLSGKKVVPVGPLVQDPVHDNEDLTIMEWLNTKGKYSTVFVSFGSEYFLSKGDLEGVAHGLELSSVNFVWVVRFPKGENIIVEEALPKGFLKRVGERGKIVNGWAPQAKILNHSSIGGFVSHCGWNSVLEGMRFGVPIIAVPMHLDQPVNARLLQEVGAGMEVVRGSTGKIHGENMAEIINQVVKGPRGEPVRKKARDLREKLELKGDEEIDEVVKELVQLCLTEDKNNGLHLEHHHHHH

SEQ ID NO: 8 - protein, 448 aa, Daucus carota subsp. sativus
MNGKRNKNLTVLMFPWLAHGHISPYLELGKKLSMRNFNVQLCSTPANLTSIRKKIGEESCIQLVQLDLPSLSNLPPCYHTTNGLPPHLMDTLKTAFDRAKPGFSKILEAVKPDLLVYDFLRPWPAEAALEQRIPAVQFIATSATMTSFMLHAFKNPSVVYPFSTIFYRGYENAQVGKSGECGELRKNIESLERSNEVIFIKGVKEMEGKFTDYLSTLSGKRVVHVGPLVQEPDSKDQTNSEIIRWLDKKKKCSTIFISFGSEYFLSKEDFEEVAHGLLLSTVNFIWVVRFPVAEKIRVEDKLPSRFLEKVGDRGRIVEGWAPQARILGHSSIGGFVSHCGWNSVIESMHFGVPIIAMPMHLDQPINARLVKEFGTGIEVLRDGDGRLEREGIASVIEQVVFKKNGRYVRKKTKKLCANIRRKGDEEIDEVVRELMQLINSLEHHHHHH

SEQ ID NO: 9 - protein, 456 aa, Catharanthus roseus
MENYRNLSVLMFPWLAHGHISPFLELAKKLSARNFTVYLCSTGATLNSVKEKLSENFKNSIFLVELPLPEFSNLPPHYHTTNGLPPELMPILKEAFNQAGPNFLEILRNLKPDLLIYDSLQPWAPKAALAMNIPAVDFITSSSVMTALMMHVFKKPGLRFPYSDSIFYHSHEASFEKRLQDKLKGHFVEKLPVIECIEQSSDIILIKGFNEFDGKYSDYLTKLTGKKVIAVGPLVQEPTIDDENENFEIIKWLNKKEKRSTVFVSFGSEYFLSKEDREEIALGLERSDVNFIFVIRFPKGENSKLEEALPKGFFKRVGERGRVLEGWAPQAKILSHVSIGAFVSHCGWSSILESMQYGVPIIALPMHLDQPINARLVAEVGAGIEVCRDVNGRIRRREVAIAVNQVMKGEIGEFVKKQVKYLQSKIEEKGDEEMDRVVEVLFQVCLKNQNKKNGFH

SEQ ID NO: 10 - protein, 457 aa, Solanum tuberosum
MDASMEINQKSIRVLMFPWLGHGHISPFFELAKKLVKRNFTIFLCSTPANFISIKQKLINENLTEKIHLVDLRLPSLPDLPPHYHTTNGLPPHLMSTLKKAFAKARPNFTQIINSIEPDLLIYDLLQPWAPKVAAEKNIPSVVFVTSSATMFSYMFHTFRYPNSVFPFSCIYYRDYELARMVKNQELEPIEQQQKDNTSVKLCFKRSSNIVLIKGFKEIDGQYCDYISSLTKKRVVPVGPLVQEPTSEDGNSQILTWLNQKSKGSTIFVSFGSEYFLSQEDREEIAHGLEKSRVNFIWVVRFPKGEKLKLEQALPRGFFKKVGERGMVVEDWAPQAKILGNPSIGGFVSHCGWNSVMESMKIGVPIIAMPMHLDQPLNARLVEEVGIGLEVVRDKDGKLDGEQISEIINKVVLDKEGESIREKAKKMSETIRVKGDEEIDDVVQELVNLCKTRSNVV

SEQ ID NO: 11 - protein, 450 aa, Solanum commersonii
MNGFTNNPLRVLMFPWLGYGHISPFLELAKKLSQRNFVIYLCSTPVILNSIKKKLSPEFSPSIHLLELHLQTLPNLPPSHHTTNGLPPHLMNTLKEAFDLASPDFALILKTLKPDLLIYDFLQPWAPKSAAELKIPAVEFISSSSTMTAYMLHEFNKPGIKFPFSSICYRDYEKARIEKQEASISVEKLEEDKRRVRECFYLSCDIVLIKSFKEIEGKYSDYITNLTGKKVVPLGPLVQEPTLEDSESELITWLNEKEKKSTIFVSFGSEYFLSNEDLVEIAYGLETSKVNFIWPIRFQKGENLELEEALPKGFFNRVGNRGKVFNGWAPQAKILEHSSIGGFVSHCGWSSVMESMKYGVPIIAMPMHIDQPINSRLVEDVGIAVEVVRDSDGKLHREEVAAIINQVVLDKDGEFLRQKAKDMKEKLCIKGDEEIEQVAKELEKLCAKFL

SEQ ID NO: 12 - protein, 454 aa, Solanum chilense
MDGSNEKSIRVLMFPWLGHGHISPFFELAKKLVKRNFTIFLVSTPANFISIKQKLIHENLCDKIHLFDLRLPSLPDLPPHYHTTNGLPPHLMSTLKKAFAKSRPIFTQIMNTIEPDLLLYDLLQPWAPKVAKEKNIPSVVFVTSSATMFSYMFHNFRYPNSEFPFSSIYYRDYELTRLIKNQEMETIEQHQRDNNSVKLCFKRSTNIVLIKGFKEIDGQYCEYISSLTKKRVVPVGPLVQEQTSEDNNSQILTWLNQKSKGSTIFVSFGSEYFLSQEDREEIAHGLEQSRVNFIWVVRFPKGEKIKLEQALPPDFFKKVGERGMVVEDWAPQAKILGNPNIGGFVSHCGWNSVLESMKIGVPIIAMPMHLDQPLNARLVEEVGMGLEVVRDKDGKLDGEQISEIINKVVLEKEGESIREKAKKMSETIRVKGDEEIDDVVQELVNLCKTRSNVV

SEQ ID NO: 13 - protein, 805 aa, Phaseolus vulgaris
MAADRLTRVHSLRERLDETLSANRNEILALLSRIEAKGTGILQHHQVIAEFEEIPEESRQKLIDGAFGEVLRSTQEAIVLPPWVALAVRPRPGVWEYLRVNVHALVVEVLQPAEYLRFKEELVDGSSNGNFVLELDFEPFTASFPRPTLNKSIGNGVQFLNRHLSAKLFHDKESLHPLLEFLRLHSVNGKTLMLNDRIQNPDALQHVLRKAEEYLGTVPPETPYSEFEHKFQEIGLERGWGANAELVLESIQLLLDLLEAPDPCTLETFLGRIPMVFNVVILSPHGYFAQDNVLGYPDTGGQVVYILDQVRALENEMLHRIKQQGLDIVPRILIITRLLPDAVGTTCGQRLEKVFGTEHSHILRVPFRTENGIVRKWISRFEVWPYLETYTEDVAHELAKELQGKPDLIVGNYSDGNIVASLLAHKLGVTQCTIAHALEKTKYPESDIYWKKLEERYHFSCQFTADLFAMNHTDFIITSTFQEIAGSKDTVGQYESHTAFTLPGLYRVVHGIDVFDPKFNIVSPGADQTIYFSHKETSRRLTSFHPEIEELLYSSVENEEHICVLKDRTKPIIFTMARLDRVKNITGLVEWYGKNEKLRELVNLVVVAGDRRKESKDLEEKAEMKKMYSLIETYKLNGQFRWISSQMNRVRNGELYRVISDTRGAFVQPAVYEAFGLTVVEAMTCGLPTFATCNGGPAEIIVHGKSGFHIDPYHGDRAADLLVEFFEKCKVEPSHWDTISQAGLQRIEEKYTWQIYSQRLLTLTGVYGFWKHVSNLDRLESRRYLEMFYALKYRKLAESVPLAVE

SEQ ID NO: 14 - protein, 800 aa, Glycine max
MATDRLTRVHSLRERLDETLTANRNEILALLSRIEAKGKGILQHHQVIAEFEEIPEENRQKLTDGAFGEVLRSTQEAIVLPPWVALAVRPRPGVWEYLRVNVHALVVEELQPAEYLHFKEELVDGSSNGNFVLELDFEPFNAAFPRPTLNKSIGNGVQFLNRHLSAKLFHDKESLHPLLEFLRLHSVKGKTLMLNDRIQNPDALQHVLRKAEEYLGTVPPETPYSEFEHKFQEIGLERGWGDNAERVLESIQLLLDLLEAPDPCTLETFLGRIPMVFNVVILSPHGYFAQDNVLGYPDTGGQVVYILDQVRALENEMLHRIKQQGLDIVPRILIITRLLPDAVGTTCGQRLEKVFGTEHSHILRVPFRTEKGIVRKWISRFEVWPYLETYTEDVAHELAKELQGKPDLIVGNYSDGNIVASLLAHKLGVTQCTIAHALEKTKYPESDIYWKKLEERYHFSCQFTADLFAMNHTDFIITSTFQEIAGSKDTVGQYESHTAFTLPGLYRVVHGIDVFDPKFNIVSPGADQTIYFPHTETSRRLTSFHPEIEELLYSSVENEEHICVLKDRSKPIIFTMARLDRVKNITGLVEWYGKNAKLRELVNLVVVAGDRRKESKDLEEKAEMKKMYGLIETYKLNGQFRWISSQMNRVRNGELYRVICDTRGAFVQPAVYEAFGLTVVEAMTCGLPTFATCNGGPAEIIVHGKSGFHIDPYHGDRAADLLVDFFEKCKLDPTHWDKISKAGLQRIEEKYTWQIYSQRLLTLTGVYGFWKHVSNLDRRESRRYLEMFYALKYRKLVCIV

SEQ ID NO: 15 - protein, 835 aa, Glycine max
MATDRLTRVHSLRERLDETLTANRNEILALLSRIEAKGKGILQHHQVIAEFEEIPEENRQKLTDGAFGEVLRSTQEAIVLPPWVALAVRPRPGVWEYLKVNVHALVVEELQPAEYLHFKEELVDGSSNGNFVLELDFEPFNAAFPRPTLNKSIGNGVQFLNRHLSAKLFHDKESLHPLLEFLRLHSVKGKTLMLNDRIQNPDALQHVLRKAEEYLGTVPPETPYSEFEHKFQEIGLERGWGDNAERVLESIQLLLDLLEAPDPCTLETFLGRIPMVFNVVILSPHGYFAQDNVLGYPDTGGQVVYILDQVRALENEMLHRIKQQGLDIVPRILIITRLLPDAIGTTCGQRLEKVFGTEHSHILRVPFRTEKGIVRQWISRFEVWPYLETYTEDVAHELAKELQGKPDLIVGNYSDGNIVASLLAHKLGVTQCTIAHALEKTKYPESDIYWKKLEERYHFSCQFTADLFAMNHTDFIITSTFQEIAGSKDTVGQYESHTAFTLPGLYRVVHGIDVFDPKFNIVSPGADQTIYFPPTETSRRLTSFHPEIEELLYSSVENEEHICVLKDRSKPIIFTMARLDRVKNITGLVEWYGKNAKLRELVNLVVVAGDRRKESKDLEEKAEMKKMYGLIETYKLNGQFRWISSQMNRVRNGELYRVICDTKGAFVQPAIYEAFGLTVVEAMTCGLPTFATCNGGPAEIIVHGKSGFHIDPYHGDRAADLLVDFFEKCKLDPTHWETISKAGLQRIEEKYTWQIYSQRLLTLTGVYGFWKHVSNLDRRESRRYLEMFYALKYRKLVPSLCPLLLSKLRMKSWIKKWRNRLFVSHLEFVLLEFYK

SEQ ID NO: 16 - protein, 805 aa, Acacia pycnantha
MASDRLTRVHSLRERLDETLTAHRNEILALLSRIEAKGKGILQHHQVIAEFEEIPEENRLKLIDGAFGEVLRSTQEAIVLPPWVALAVRPRPGVWEYLRVNVHALVVEELRVAEYLRFKEELVDGSANGNFVLELDFEPFTASFPRPTLNKSIGNGVEFLNRHLSAKMFHDKESMHPLLEFLRLHSVKGKTLMLNDRIQNLNSLQHVLRKAEDYLGTVPPQTPYSEFEHKFQEIGLERGWGDNAERVLEMIQLLLDLLEAPDPCTLETFLGRIPMVFNVVILSPHGYFAQDNVLGYPDTGGQVVYILDQVRALENEMLQRIKHQGLDIIPRILIITRLLPDAAGTTCGQRLEKVYGTEHCHILRVPFRDEKGMVRKWISRFEVWPYLETYTEDVAHELSKELQGKPDLIIGNYSDGNIVASLLAHKLGVTQCTIAHALEKTKYPDSDIYWKKFEDKYHFSSQFTADLFAMNHTDFIITSTFQEIAGSKDTVGQYESHTAFTLPGLYRVVHGIDVFDPKFNIVSPGADMDIYFPFTETKRRLTSFQPEIEELLYSSVENEEHICVLKDRSKPIIFTMARLDRVKNITGLVEWYGKNARLRELVNLVVVAGDRRKESKDLEEKAEMKKMYGLIETYKLNGQFRWISSQMNRVRNGELYRVIGDTKGAFVQPALYEAFGLTVVEAMTCGLPTFATCNGGPAEIIVNGKSGFHIDPYHGDRAAEILVDFFEKCKVDPSHWDNISQGGLQRIHEKYTWQIYSQRLLTLTGVYGFWKHVSNLDRRESRRYLEMFYALKYRKLAESVPLAIE

SEQ ID NO: 17 - protein, 805 aa, Vigna radiata
MATDRLTRVHSLRERLDETLSANRNEILALLSRIEGKGKGILQHHQVIAEFEEIPEESRQKLTDGAFGEVLRSTQEAIVLPPWVALAVRPRPGVWEYLRVNVHALVVEVLQPAEYLRFKEELVDGSSNGNFVLELDFEPFTASFPRPTLNKSIGNGVQFLNRHLSAKLFHDKESLHPLLEFLRLHSVKGKTLMLNDRIQNPDALQHVLRKAEEYLGTVPPETPYSAFEHKFQEIGLERGWGDNAERVLESIQLLLDLLEAPDPCTLETFLGRIPMVFNVVILSPHGYFAQDNVLGYPDTGGQVVYILDQVRALENEMLHRIKQQGLDIVPRILIITRLLPDAVGTTCGQRLEKVFGTEHSHILRVPFRTENGIVRKWISRFEVWPYLETYTEDVAHELAKELQGKPDLIVGNYSDGNIVASLLAHKLGVTQCTIAHALEKTKYPESDIYWKKLEERYHFSCQFTADLFAMNHTDFIITSTFQEIAGSKDTVGQYESHTAFTLPGLYRVVHGIDVFDPKFNIVSPGADQTIYFPHTETSRRLTSFHTEIEELLYSSVENEEHICVLKDRSKPIIFTMARLDRVKNITGLVEWYGKNAKLRELVNLVVVAGDRRKESKDLEEKAEMKKMYSLIETYKLNGQFRWISSQMNRVRNGELYRVIADTKGAFVQPAVYEAFGLTVVEAMTCGLPTFATCNGGPAEIIVHGKSGFHIDPYHGDRAADLLVEFFEKVKVDPSHWDKISQAGLQRIEEKYTWQIYSQRLLTLTGVYGFWKHVSNLDRRESRRYLEMFYALKYRKLAESVPLAVE

SEQ ID NO: 18 - protein, 804 aa, Trifolium subterraneum
MAGLTRVHSLRERLDETLTANRNEILALLSRIEAKGKGILQHHQIIAEFEEIPEESRQKLSDGAFGEVLRSTQEAIVLPPWVALAVRPRPGVWEYLRVNVHALVVENLQPAEFLKFKEELVDGSANGNFVLELDFEPFTASFPRPTLNKSIGNGVQFLNRHLSAKLFHDKESLHPLLEFLRLHSYEGKTLMLNDRVQNPDSLQHVLRKAEEYLGTVAPETPYSEFEHKFQEIGLERGWGATADRVLESIQLLLDLLEAPDPCTLETFLDRIPMVFNVVILSPHGYFAQDDVLGYPDTGGQVVYILDQVRALENEMLLRIKQQGLDIIPRILIITRLLPDAVGTTCGQRLEKVYGTEHCHILRVPFRDSKGIVRKWISRFEVWPYLETYTEDVAHELAKELHGKPDLIVGNYSDGNIVASLLAHKLGVTQCTIAHALEKTKYPESDIYWKKFEEKYHFSCQFTADLFAMNHTDFIITSTFQEIAGSKDTVGQYESHTAFTLPGLYRVVHGIDVFDPKFNIVSPGADPTIYFPYTETSRRLTSFHPEIEELLYSSVENTEHICVLKDRNKPIIFTMARLDRVKNITGLVEWYGKNAKLRELVNLVVVAGDRRKESKDLEEIAEMKKMYGLIETYKLNGQFRWISSQMNRVRNGELYRVICDTKGAFVQPAVYEAFGLTVVEAMATGLPTFATLNGGPAEIIVHGKSGFHIDPYHGDRAADLLVEFFEKCKVDPSHWDTISHGGLQRIEEKYTWRIYSQRLLTLTGVYGFWKHVSNLDRLESRRYLEMFYALKYRKLAESVPLAVEE

SEQ ID NO: 19 - protein, 806 aa, Vigna angularis
MAHHPLTHSHAFRERIDETLSGNRNEILALLSRLEAKGKGILQHHQVIAEFEEIPEENRKKLQDGAFGEVLRSTQEAIVLPPFVALAVRPRPGVWEYLRVNLHMLVVDELRPAEYLRFKEELVEGTANGNFVLELDFEPFNASFPRPTLNKSIGNGVEFLNRHLSAKLFHDKESMQPLLEFLRLHSYKGTTMMLNDKVQNLNSLQHVLRKAEEYLTSVAPATPYSEFESRFQEIGLERGWGDTAERVLEMIQLLLDLLEAPDPCTLETFLGRVPMVFNVVILSPHGYFAQDNVLGYPDTGGQVVYILDQVRALENEMLNRIKKQGLDITPRILIITRLLPDAVGTTCGERLERVYDTEYCDILRVPFRTEKGIVRKWISRFEVWPYLETYAEDVAVELAKELQAKPDLIVGNYSDGNIVASLLAHKLGVTQCTIAHALEKTKYPESDIYWKKFEEKYHFSCQFTADLFAMNHTDFIITSTFQEIAGSKDTVGQYESHTAFTLPGLYRVVHGIDVFDPKFNIVSPGADMGIYFPYTETERRLTNFHPEIEELLYSSVENEEHICVLKDRNKPIIFTMARLDRVKNITGLVEWYGKNARLRELVNLVVVAGDRRKESKDLEEKAEMKKMYGLIETYKLNGQFRWISSQMNRVRNGELYRVICDTKGAFVQPAVYEAFGLTVVEAMTCGLPTFATFNGGPAEIIVHGKSGYHIDPYHGDRAAEILVDFFEKSKADPSHWDKISEGGLKRIQEKYTWQIYSDRLLTLTGVYGFWKHVTNLERRESKRYLEMFYALKYRKLAESVPLAIEE

SEQ ID NO: 20 - protein, 806 aa, Cannabis sativa
MPERALTRVHSLRERLDETLSAHRNEIVALLSRIEAKGKGFLQPHQIIAEFEAIPEVNRKKLLDGAFGEVLRATQEAICLPPWVALAVRPRPGVWEYIRVNVHALVIEELQVSEYLHFKEELVDGSANGNFVLELDFEPFNASFPRPTLSKSIGNGVEFLNRHLSAKLFHDKESMHPLLEFLRVHCYKGKNMMLNDRIHNLNGLQHVLRKAEEYLTSLAPETPYAEFEHKFQEIGLERGWGDTAERVLEMIQLLLDLLEAPDPCTLEKFLGRIPMVFNVVILSPHGYFAQDNVLGYPDTGGQVVYILDQVRALENEMLLRIKQQGLDIKPRILIITRLLPDAVGTTCGQRLEKVYDTEHTHILRVPFRDEKGMVRKWISRFEVWPYLETYTEDVAHELAKELQGKPDLIIGNYSDGNIVASLLAHKLGVTQCTIAHALEKTKYPDSDIYWKKLEEKYHFSCQFTADLIAMNHTDFIITSTFQEIAGSKDTVGQYESHTAFTLPGLYRVVHGIDVFDPKFNIVSPGADMSIYFPYTETEKRLTYFHPEIEELLYSDVENEEHICVLKDRNKPIIFTMARLDRVKNITGLVEWYGKNKKLRELVNLVVVAGDRRKESKDIEEKAEMAKMYGLIETYKLNGQFRWISSQMNRVRNGELYRYICDTKGAFVQPAVYEAFGLTVVEAMTCGLPTFATCKGGPAEIIVHGKSGYHIDPYHGDRAAETLVEFFEKCKVDPSHWDKISEGGLQRIYEKYTWKIYSERLLTLTGVYGFWKHVSNLDHQESRRYLEMFYALKYRKLAESVPLAVDE